European Patent Specification EP 3 920 107 B1, published February 11, 2026. Title: NANO COMPUTING DEVICE AND METHOD OF OPERATING NANO COMPUTING DEVICE. Applicant: Seoul National University R&DB Foundation. The sequence listing filed with the application follows.

SEQUENCE LISTING (50 sequences)

SEQ ID NO: 1 - DNA, 39 bp, Artificial Sequence
  Synthetic
aaaaaaaaaaaaaaaaactgccattcatttaccgtctac

SEQ ID NO: 2 - DNA, 39 bp, Artificial Sequence
  Synthetic
aaaaaaaaaaaaaaataaacccatgctaaccgctaacac

SEQ ID NO: 3 - DNA, 39 bp, Artificial Sequence
  Synthetic
aaaaaaaaaaaaaaatcttaaagtcccgtcacagtctac

SEQ ID NO: 4 - DNA, 39 bp, Artificial Sequence
  Synthetic
aaaaaaaaaaaaaaaaccaaagacccaagatactcgcac

SEQ ID NO: 5 - DNA, 39 bp, Artificial Sequence
  Synthetic
aaaaaaaaaaaaaaacgcactaagacgaattcacttttc

SEQ ID NO: 6 - DNA, 75 bp, Artificial Sequence
  Synthetic
aaaaaaaaaaaaaaaataacgagcatcgaacttacatcgcgttactacactgtcactgatcatcgcatgctatac

SEQ ID NO: 7 - DNA, 39 bp, Artificial Sequence
  Synthetic
cacaacatagaatcacgtacataaaaaaaaaaaaaaaaa

SEQ ID NO: 8 - DNA, 39 bp, Artificial Sequence
  Synthetic
ccgttctacaaatcaaagcgcatcaaaaaaaaaaaaaaa

SEQ ID NO: 9 - DNA, 39 bp, Artificial Sequence
  Synthetic
ctcgtcactctagcacaatctcgaaaaaaaaaaaaaaaa

SEQ ID NO: 10 - DNA, 39 bp, Artificial Sequence
  Synthetic
cataatctataatcatcctcataaaaaaaaaaaaaaaaa

SEQ ID NO: 11 - DNA, 49 bp, Artificial Sequence
  Synthetic
ctctctgcctcgttcagacaaaactcatcctactaaaaaaaaaaaaaaa

SEQ ID NO: 12 - DNA, 39 bp, Artificial Sequence
  Synthetic
caataacgacaaactaattcagcaaaaaaaaaaaaaaaa

SEQ ID NO: 13 - DNA, 75 bp, Artificial Sequence
  Synthetic
ctctctgcctcgttcagacaaaactcatcctactcgatactttctgtaacttttccttaaaaaaaaaaaaaaaaa

SEQ ID NO: 14 - DNA, 38 bp, Artificial Sequence
  Synthetic
ttatgtacgtgattctatgttgtggattgttttctagg

SEQ ID NO: 15 - DNA, 38 bp, Artificial Sequence
  Synthetic
gatgcgctttgatttgtagaacgggataggcgacatag

SEQ ID NO: 16 - DNA, 38 bp, Artificial Sequence
  Synthetic
tcgagattgtgctagagtgacgaggatgtcagggacag

SEQ ID NO: 17 - DNA, 38 bp, Artificial Sequence
  Synthetic
ttatgaggatgattatagattatggtatttagaaaatg

SEQ ID NO: 18 - DNA, 32 bp, Artificial Sequence
  Synthetic
cgttattgaatccttagagaaaagtgaattcg

SEQ ID NO: 19 - DNA, 38 bp, Artificial Sequence
  Synthetic
gattctatgttgtgccttcattaagtagacggtaaatg

SEQ ID NO: 20 - DNA, 38 bp, Artificial Sequence
  Synthetic
cctagaaaacaatctctcgtattcgtagacggtaaatg

SEQ ID NO: 21 - DNA, 38 bp, Artificial Sequence
  Synthetic
gatttgtagaacggatatcattacgtagacggtaaatg

SEQ ID NO: 22 - DNA, 38 bp, Artificial Sequence
  Synthetic
ctatgtcgcctatccatatacagcgtagacggtaaatg

SEQ ID NO: 23 - DNA, 38 bp, Artificial Sequence
  Synthetic
gctagagtgacgagaagatataccgtagacggtaaatg

SEQ ID NO: 24 - DNA, 38 bp, Artificial Sequence
  Synthetic
ctgtccctgacatcttcttatctcgtagacggtaaatg

SEQ ID NO: 25 - DNA, 38 bp, Artificial Sequence
  Synthetic
gattatagattatgcctacgtctagtagacggtaaatg

SEQ ID NO: 26 - DNA, 38 bp, Artificial Sequence
  Synthetic
cattttctaaatacacagctaacagtagacggtaaatg

SEQ ID NO: 27 - DNA, 38 bp, Artificial Sequence
  Synthetic
gattctatgttgtgttctttaccagtgttagcggttag

SEQ ID NO: 28 - DNA, 38 bp, Artificial Sequence
  Synthetic
cctagaaaacaatctatgcctactgtgttagcggttag

SEQ ID NO: 29 - DNA, 38 bp, Artificial Sequence
  Synthetic
gatttgtagaacggaacattaccagtgttagcggttag

SEQ ID NO: 30 - DNA, 38 bp, Artificial Sequence
  Synthetic
ctatgtcgcctatcttaaaccgtagtgttagcggttag

SEQ ID NO: 31 - DNA, 38 bp, Artificial Sequence
  Synthetic
gctagagtgacgagataccaaatagtgttagcggttag

SEQ ID NO: 32 - DNA, 38 bp, Artificial Sequence
  Synthetic
ctgtccctgacatcactactatttgtgttagcggttag

SEQ ID NO: 33 - DNA, 38 bp, Artificial Sequence
  Synthetic
gattatagattatgacagtcgcaggtgttagcggttag

SEQ ID NO: 34 - DNA, 38 bp, Artificial Sequence
  Synthetic
cattttctaaataccacggccttggtgttagcggttag

SEQ ID NO: 35 - DNA, 38 bp, Artificial Sequence
  Synthetic
gattctatgttgtgagcttcatgcgtagactgtgacgg

SEQ ID NO: 36 - DNA, 38 bp, Artificial Sequence
  Synthetic
cctagaaaacaatctccagtctttgtagactgtgacgg

SEQ ID NO: 37 - DNA, 38 bp, Artificial Sequence
  Synthetic
gatttgtagaacggaacctagtaagtagactgtgacgg

SEQ ID NO: 38 - DNA, 38 bp, Artificial Sequence
  Synthetic
ctatgtcgcctatctaaccttacagtagactgtgacgg

SEQ ID NO: 39 - DNA, 38 bp, Artificial Sequence
  Synthetic
gctagagtgacgagcttgcaaacagtagactgtgacgg

SEQ ID NO: 40 - DNA, 38 bp, Artificial Sequence
  Synthetic
ctgtccctgacatctaatcaagcagtagactgtgacgg

SEQ ID NO: 41 - DNA, 38 bp, Artificial Sequence
  Synthetic
gattatagattatgaacctagtaagtagactgtgacgg

SEQ ID NO: 42 - DNA, 38 bp, Artificial Sequence
  Synthetic
cattttctaaatactaaccttacagtagactgtgacgg

SEQ ID NO: 43 - DNA, 38 bp, Artificial Sequence
  Synthetic
gattctatgttgtgttacaataacgtgcgagtatcttg

SEQ ID NO: 44 - DNA, 38 bp, Artificial Sequence
  Synthetic
cctagaaaacaatctatcacacaggtgcgagtatcttg

SEQ ID NO: 45 - DNA, 38 bp, Artificial Sequence
  Synthetic
gatttgtagaacggacactttgcggtgcgagtatcttg

SEQ ID NO: 46 - DNA, 38 bp, Artificial Sequence
  Synthetic
ctatgtcgcctatccaaatagaatgtgcgagtatcttg

SEQ ID NO: 47 - DNA, 38 bp, Artificial Sequence
  Synthetic
gctagagtgacgagatatcacaaggtgcgagtatcttg

SEQ ID NO: 48 - DNA, 38 bp, Artificial Sequence
  Synthetic
ctgtccctgacatctacttacgatgtgcgagtatcttg

SEQ ID NO: 49 - DNA, 38 bp, Artificial Sequence
  Synthetic
gattatagattatgacactttgcggtgcgagtatcttg

SEQ ID NO: 50 - DNA, 38 bp, Artificial Sequence
  Synthetic
cattttctaaataccaaatagaatgtgcgagtatcttg